European Patent Application EP 4 692 348 A1, published February 11, 2026. Title: ARTIFICIAL RNAS FOR TREATING REPEAT EXPANSION DISORDERS. Applicant: NOCTURNA THERAPEUTICS SL. The sequence listing filed with the application follows.

SEQUENCE LISTING (91 sequences)

SEQ ID NO: 1 - RNA, 289 nt, synthetic construct
  source 1..289: mol_type = other RNA
cccggttccgcacggtggtagtagcagcattcttggctatgggtggtggttctctatactcggtagcagtagcagcatttttggttataggcccagctgagacaagggcggtggcagcggtagcatttccggttataagtttaagtttgcactgcccggcagtagtggtagcattttcggttgtgaacaccatcgccccccatgcagcagcagtagcagcattctcggttacagaactaaggcacccacttatggtagcagcagcagcattcccggctatgagacagtc

SEQ ID NO: 2 - RNA, 289 nt, synthetic construct
  source 1..289: mol_type = other RNA
cccggttccgcaatggtctgtgattttctcggcagcggcagtcgtggtggttctctatacgtggtctgtgatcctcccagtagtggcagttgcccagctgagacaaggatggtctgtggtcttcccagcagtggcagtggtttaagtttgcactgcatggtttgtgatcctcttagcagtagcggtcacaccatcgccccccatgtggtctgtggttctcccggcagcagtagcgaactaaggcacccctccatggtttgtggttttcctagtagtagcagtgacagtc

SEQ ID NO: 3 - RNA, 289 nt, synthetic construct
  source 1..289: mol_type = other RNA
cccggttccgcacagtagcagtagtggtgttctcggctataacgtggtggttctctataccagcggtagcggtagcgtttttggctgcaatgcccagctgagacaaggcagcggtggcagcagcatttctggttacaaggtttaagtttgcactgccagtagtagcagtagcattcccggctgtaacacaccatcgccccccatcagtagcggcggcggcgtttctggctacaagaactaaggcaccgacaacagcagcagcggtggtgtttttggctacaagacagtc

SEQ ID NO: 4 - RNA, 289 nt, synthetic construct
  source 1..289: mol_type = other RNA
cccggttccgcaatggtctgtgatccccttagtagtagtggcgtggtggttctctatactatggtttgtggttctcccggtggtagtggcgcccagctgagacaagggatggtttgtgatttctccagtagtagtggcgtttaagtttgcactgccatggtttgtgattcctttagtggcagcagcacaccatcgccccccatgatggtctgtgatctctccggtagcagcagcaactaaggcacccatgtcatggtctgtggtctttctagcagtggtggcgacagtc

SEQ ID NO: 5 - RNA, 276 nt, synthetic construct
  source 1..276: mol_type = other RNA
cccggttccgcaagcggtagcagtagtagtagcatggggataagtattggcctttaccgagcagtagtggcggcggtagtaaaacactgtccattaagtcactgttagtagtagcggtggcagcagtaagacgcccgcttaaacgtctttggtagcggcggtagcggcagcagcacctgtcgtcgatgagcagctgctagagcagcagcagcagcggtagtaagccaacaagagaaaaacacccataagcagtggtggtagtagcagcagacagtc

SEQ ID NO: 6 - RNA, 289 nt, synthetic construct
  source 1..289: mol_type = other RNA
cccggttccgcacagcggcagcagcagcatttccggctgcaatggtggttctctatactgatggtttgtgatctctctagtagcggtagccccagctgagacaaggggcagtagcagtagtagtattctcggttacaatttaagtttgcactgccaatggtctgtgattctttcagtggcagtggccaccatcgccccccatgacagtagtagtagtggtattcctggttgcaaactaaggcaccgaacacaatggtctgtgatcccctcagcagcagtggcgacagtc

SEQ ID NO: 7 - RNA, 265 nt, synthetic construct
  source 1..265: mol_type = other RNA
cccggttccgcaatggtctgtgatttctttggcagtagtggccgtggtggttctctatacagcggtagcagtagcagcagcgtgcccagctgagacaaggatggtctgtgatcctttcggtagtagtggcggtttaagtttgcactgcggcagtagtagtggcagtagcgcacaccatcgccccccatatggtttgtggttcctctagtagtggcagcgaactaaggcacctatagagtggcagcagtggtagcagtagacagtc

SEQ ID NO: 8 - RNA, 273 nt, synthetic construct
  source 1..273: mol_type = other RNA
cccggttccgcacagtggtagtagtagcatttctggttgtgacgtggtggttctctatacatggtttgtggttcccttagtggcggtagctgcccagctgagacaaggagtggtggcggcggcggcagtaggtttaagtttgcactgccagtagcggtggtagtatttttggttgtaacacaccatcgccccccatatggtttgtgatttctctggtggcagtggcgaactaaggcacaactccggtagtagtggtagtggtagtagacagtc

SEQ ID NO: 9 - RNA, 30 nt, synthetic construct
  source 1..30: mol_type = other RNA
cggtggtagtagcagcattcttggctatgg

SEQ ID NO: 10 - RNA, 30 nt, synthetic construct
  source 1..30: mol_type = other RNA
cggtagcagtagcagcatttttggttatag

SEQ ID NO: 11 - RNA, 30 nt, synthetic construct
  source 1..30: mol_type = other RNA
cggtggcagcggtagcatttccggttataa

SEQ ID NO: 12 - RNA, 30 nt, synthetic construct
  source 1..30: mol_type = other RNA
cggcagtagtggtagcattttcggttgtga

SEQ ID NO: 13 - RNA, 30 nt, synthetic construct
  source 1..30: mol_type = other RNA
cagcagcagtagcagcattctcggttacag

SEQ ID NO: 14 - RNA, 30 nt, synthetic construct
  source 1..30: mol_type = other RNA
tggtagcagcagcagcattcccggctatga

SEQ ID NO: 15 - RNA, 30 nt, synthetic construct
  source 1..30: mol_type = other RNA
cagtagcagtagtggtgttctcggctataa

SEQ ID NO: 16 - RNA, 30 nt, synthetic construct
  source 1..30: mol_type = other RNA
cagcggtagcggtagcgtttttggctgcaa

SEQ ID NO: 17 - RNA, 30 nt, synthetic construct
  source 1..30: mol_type = other RNA
cagcggtggcagcagcatttctggttacaa

SEQ ID NO: 18 - RNA, 30 nt, synthetic construct
  source 1..30: mol_type = other RNA
cagtagtagcagtagcattcccggctgtaa

SEQ ID NO: 19 - RNA, 30 nt, synthetic construct
  source 1..30: mol_type = other RNA
cagtagcggcggcggcgtttctggctacaa

SEQ ID NO: 20 - RNA, 30 nt, synthetic construct
  source 1..30: mol_type = other RNA
cagcagcagcggtggtgtttttggctacaa

SEQ ID NO: 21 - RNA, 30 nt, synthetic construct
  source 1..30: mol_type = other RNA
atggtctgtgattttctcggcagcggcagt

SEQ ID NO: 22 - RNA, 30 nt, synthetic construct
  source 1..30: mol_type = other RNA
gtggtctgtgatcctcccagtagtggcagt

SEQ ID NO: 23 - RNA, 30 nt, synthetic construct
  source 1..30: mol_type = other RNA
atggtctgtggtcttcccagcagtggcagt

SEQ ID NO: 24 - RNA, 30 nt, synthetic construct
  source 1..30: mol_type = other RNA
atggtttgtgatcctcttagcagtagcggt

SEQ ID NO: 25 - RNA, 30 nt, synthetic construct
  source 1..30: mol_type = other RNA
gtggtctgtggttctcccggcagcagtagc

SEQ ID NO: 26 - RNA, 30 nt, synthetic construct
  source 1..30: mol_type = other RNA
atggtttgtggttttcctagtagtagcagt

SEQ ID NO: 27 - RNA, 30 nt, synthetic construct
  source 1..30: mol_type = other RNA
atggtctgtgatccccttagtagtagtggc

SEQ ID NO: 28 - RNA, 30 nt, synthetic construct
  source 1..30: mol_type = other RNA
atggtttgtggttctcccggtggtagtggc

SEQ ID NO: 29 - RNA, 30 nt, synthetic construct
  source 1..30: mol_type = other RNA
atggtttgtgatttctccagtagtagtggc

SEQ ID NO: 30 - RNA, 30 nt, synthetic construct
  source 1..30: mol_type = other RNA
atggtttgtgattcctttagtggcagcagc

SEQ ID NO: 31 - RNA, 30 nt, synthetic construct
  source 1..30: mol_type = other RNA
atggtctgtgatctctccggtagcagcagc

SEQ ID NO: 32 - RNA, 30 nt, synthetic construct
  source 1..30: mol_type = other RNA
atggtctgtggtctttctagcagtggtggc

SEQ ID NO: 33 - RNA, 22 nt, synthetic construct
  source 1..22: mol_type = other RNA
agcggtagcagtagtagtagca

SEQ ID NO: 34 - RNA, 22 nt, synthetic construct
  source 1..22: mol_type = other RNA
agcagtagtggcggcggtagta

SEQ ID NO: 35 - RNA, 22 nt, synthetic construct
  source 1..22: mol_type = other RNA
agtagtagcggtggcagcagta

SEQ ID NO: 36 - RNA, 22 nt, synthetic construct
  source 1..22: mol_type = other RNA
agcggcggtagcggcagcagca

SEQ ID NO: 37 - RNA, 22 nt, synthetic construct
  source 1..22: mol_type = other RNA
agcagcagcagcagcggtagta

SEQ ID NO: 38 - RNA, 22 nt, synthetic construct
  source 1..22: mol_type = other RNA
agcagtggtggtagtagcagca

SEQ ID NO: 39 - RNA, 30 nt, synthetic construct
  source 1..30: mol_type = other RNA
cagcggcagcagcagcatttccggctgcaa

SEQ ID NO: 40 - RNA, 30 nt, synthetic construct
  source 1..30: mol_type = other RNA
atggtttgtgatctctctagtagcggtagc

SEQ ID NO: 41 - RNA, 30 nt, synthetic construct
  source 1..30: mol_type = other RNA
cagtagcagtagtagtattctcggttacaa

SEQ ID NO: 42 - RNA, 30 nt, synthetic construct
  source 1..30: mol_type = other RNA
atggtctgtgattctttcagtggcagtggc

SEQ ID NO: 43 - RNA, 30 nt, synthetic construct
  source 1..30: mol_type = other RNA
cagtagtagtagtggtattcctggttgcaa

SEQ ID NO: 44 - RNA, 30 nt, synthetic construct
  source 1..30: mol_type = other RNA
atggtctgtgatcccctcagcagcagtggc

SEQ ID NO: 45 - RNA, 30 nt, synthetic construct
  source 1..30: mol_type = other RNA
atggtctgtgatttctttggcagtagtggc

SEQ ID NO: 46 - RNA, 22 nt, synthetic construct
  source 1..22: mol_type = other RNA
agcggtagcagtagcagcagcg

SEQ ID NO: 47 - RNA, 30 nt, synthetic construct
  source 1..30: mol_type = other RNA
atggtctgtgatcctttcggtagtagtggc

SEQ ID NO: 48 - RNA, 22 nt, synthetic construct
  source 1..22: mol_type = other RNA
ggcagtagtagtggcagtagcg

SEQ ID NO: 49 - RNA, 30 nt, synthetic construct
  source 1..30: mol_type = other RNA
atggtttgtggttcctctagtagtggcagc

SEQ ID NO: 50 - RNA, 22 nt, synthetic construct
  source 1..22: mol_type = other RNA
agtggcagcagtggtagcagta

SEQ ID NO: 51 - RNA, 30 nt, synthetic construct
  source 1..30: mol_type = other RNA
cagtggtagtagtagcatttctggttgtga

SEQ ID NO: 52 - RNA, 30 nt, synthetic construct
  source 1..30: mol_type = other RNA
atggtttgtggttcccttagtggcggtagc

SEQ ID NO: 53 - RNA, 22 nt, synthetic construct
  source 1..22: mol_type = other RNA
agtggtggcggcggcggcagta

SEQ ID NO: 54 - RNA, 30 nt, synthetic construct
  source 1..30: mol_type = other RNA
cagtagcggtggtagtatttttggttgtaa

SEQ ID NO: 55 - RNA, 30 nt, synthetic construct
  source 1..30: mol_type = other RNA
atggtttgtgatttctctggtggcagtggc

SEQ ID NO: 56 - RNA, 22 nt, synthetic construct
  source 1..22: mol_type = other RNA
ggtagtagtggtagtggtagta

SEQ ID NO: 57 - DNA, 21 bp, synthetic construct
  source 1..21: mol_type = other DNA
gctgcccaataccaggtcaac

SEQ ID NO: 58 - DNA, 22 bp, synthetic construct
  source 1..22: mol_type = other DNA
tggtgggagaaatgctgtatgc

SEQ ID NO: 59 - DNA, 23 bp, synthetic construct
  source 1..23: mol_type = other DNA
tcctttaccaaagagacaagcac

SEQ ID NO: 60 - DNA, 24 bp, synthetic construct
  source 1..24: mol_type = other DNA
ctcaatgcagattcttggcattcc

SEQ ID NO: 61 - DNA, 24 bp, synthetic construct
  source 1..24: mol_type = other DNA
acacccacaaccggaatgagcctg

SEQ ID NO: 62 - DNA, 22 bp, synthetic construct
  source 1..22: mol_type = other DNA
ggacttggcttttcggctgctg

SEQ ID NO: 63 - DNA, 30 bp, synthetic construct
  source 1..30: mol_type = other DNA
cagcagcagcagcagcagcagcagcagcag

SEQ ID NO: 64 - RNA, 129 nt, synthetic construct
  source 1..129: mol_type = other RNA
cccggttccgcacatatgaagatagaccagcagcagcagcagcattcccggctacaactctatcccgtctcgctcgaatggtctgtgatccccccagcagcagcagcattttctcgattcgtgacagtc

SEQ ID NO: 65 - RNA, 116 nt, synthetic construct
  source 1..116: mol_type = other RNA
cccggttccgcatagttaaaaaatccacagcagcagcagcattcccggctacaacagagtacaacttgatcgaccagcagcagcagcagcagcaagaaaaaatagtggagacagtc

SEQ ID NO: 66 - RNA, 116 nt, synthetic construct
  source 1..116: mol_type = other RNA
cccggttccgcaagttgattgatatcacagcagcagcagcagcagcataaactagcgtgacgatgctcagcagcagcagcattcccggctacaactcctcgctcttctggacagtc

SEQ ID NO: 67 - DNA, 119 bp, synthetic construct
  source 1..119: mol_type = other DNA
cccggttccgcagcgagtgtcgttgagatggtctgtgatccccccagcagcagcagccccatgtatggacccactaacagcagcagcagcagcagcaatggaacagagctgtgacagtc

SEQ ID NO: 68 - RNA, 119 nt, synthetic construct
  source 1..119: mol_type = other RNA
cccggttccgcatctccaacgatggtacagcagcagcagcagcagcatcacctatgtgccgacttaaatggtctgtgatccccccagcagcagcagctttcgtgaggacttcgacagtc

SEQ ID NO: 69 - RNA, 166 nt, synthetic construct
  source 1..166: mol_type = other RNA
cccggttccgcatactgaaggattttacagcagcagcagcattcccggctacaacctgacaatcaccaacgcaaatggtctgtgatccccccagcagcagcagctttgatatagcggacaaaaacagcagcagcagcagcagcaaaaaaatcataaggcgacagtc

SEQ ID NO: 70 - RNA, 202 nt, synthetic construct
  source 1..202: mol_type = other RNA
cccggttttccgcattcttattccagacttttttccagcagcagcagcagcagcaccgcaggttccttcgcacaacttcagcagcagcagcattttcccggcttacaacttttttttattaccttattcattagcttattggttcttgttgattccccccagcagcagcagcttttttttccttgattccacttgacagttc

SEQ ID NO: 71 - RNA, 166 nt, synthetic construct
  source 1..166: mol_type = other RNA
cccggttccgcatcaatgcatcctatccagcagcagcagcagcagcaccgcatgctaatatccctccatggtctgtgatccccccagcagcagcagccttattgtcgcatagtctcccagcagcagcagcattcccggctacaattttccgactcatacgacagtc

SEQ ID NO: 72 - RNA, 193 nt, synthetic construct
  source 1..193: mol_type = other RNA
cccggttttccgcaattattttcaattaacgaacagcagcagcagcagcagcacaagattccttcaccttaattgcaattggttcttgttgattccccccagcagcagcagcttgagttcccgagcaattaggcgcagcagcagcagcattttcccggcttacaattgaattattgcaggttgttgacagttc

SEQ ID NO: 73 - RNA, 27 nt, synthetic construct
  source 1..27: mol_type = other RNA
cagcagcagcagcattcccggctacaa

SEQ ID NO: 74 - RNA, 30 nt, synthetic construct
  source 1..30: mol_type = other RNA
atggtctgtgatccccccagcagcagcagc

SEQ ID NO: 75 - RNA, 19 nt, synthetic construct
  source 1..19: mol_type = other RNA
agcagcagcagcagcagca

SEQ ID NO: 76 - RNA, 30 nt, synthetic construct
  source 1..30: mol_type = other RNA
ttgtagccgggaatgctgctgctgctgctg

SEQ ID NO: 77 - RNA, 30 nt, synthetic construct
  source 1..30: mol_type = other RNA
gctgctgctgctggggggatcacagaccat

SEQ ID NO: 78 - RNA, 22 nt, synthetic construct
  source 1..22: mol_type = other RNA
tgctgctgctgctgctgctgct

SEQ ID NO: 79 - RNA, 184 nt, synthetic construct
  source 1..184: mol_type = other RNA
ttgtagccgggaatgctgctgctgctgctgctgctgctgctgctgctgctgctgctgctgctgctgctgctgctggggggatcacagaccatttgtagccgggaatgctgctgctgctgctgctgctgctgctgctgctgctgctgctgctgctgctgctgctgctggggggatcacagaccat

SEQ ID NO: 80 - RNA, 92 nt, synthetic construct
  source 1..92: mol_type = other RNA
ttgtagccgggaatgctgctgctgctgctgctgctgctgctgctgctgctgctgctgctgctgctgctgctgctggggggatcacagaccat

SEQ ID NO: 81 - RNA, 30 nt, synthetic construct; identical to SEQ ID NO: 76
  source 1..30: mol_type = other RNA

SEQ ID NO: 82 - RNA, 30 nt, synthetic construct
  source 1..30: mol_type = other RNA
cggcagcggcggcggcattcccggctacga

SEQ ID NO: 83 - RNA, 30 nt, synthetic construct
  source 1..30: mol_type = other RNA
cagcagcggcggcggcattcccggctacga

SEQ ID NO: 84 - RNA, 30 nt, synthetic construct
  source 1..30: mol_type = other RNA
cagtagcggcggcggcattcccggctacga

SEQ ID NO: 85 - RNA, 30 nt, synthetic construct
  source 1..30: mol_type = other RNA
cggtagcggcggcggcattcccggctacga

SEQ ID NO: 86 - RNA, 30 nt, synthetic construct
  source 1..30: mol_type = other RNA
cagcggcggcggcggcattcccggctacga

SEQ ID NO: 87 - RNA, 30 nt, synthetic construct
  source 1..30: mol_type = other RNA
cggcggcggcggcggcattcccggctacga

SEQ ID NO: 88 - RNA, 30 nt, synthetic construct
  source 1..30: mol_type = other RNA
cagtggcggcggcggcattcccggctacga

SEQ ID NO: 89 - RNA, 30 nt, synthetic construct
  source 1..30: mol_type = other RNA
cggtggcggcggcggcattcccggctacga

SEQ ID NO: 90 - RNA, 30 nt, synthetic construct
  source 1..30: mol_type = other RNA
cagcagtggcggcggcattcccggctacga

SEQ ID NO: 91 - RNA, 30 nt, synthetic construct
  source 1..30: mol_type = other RNA
cggcagtggcggcggcattcccggctacga